European Patent Specification EP 4 623 103 B1, published February 4, 2026. Title: METHODS FOR OBTAINING CORRECTLY ASSEMBLED NUCLEIC ACIDS. Applicant: DNA Script. Application EP. The sequence listing filed with the application follows.

SEQUENCE LISTING (18 sequences)

SEQ ID NO: 1 - DNA, 20 bp, synthetic construct
  source 1..20: mol_type = other DNA
aatgatacggcgaccaccga

SEQ ID NO: 2 - DNA, 24 bp, synthetic construct
  source 1..24: mol_type = other DNA
caagcagaagacggcatacgagat

SEQ ID NO: 3 - DNA, 33 bp, synthetic construct
  source 1..33: mol_type = other DNA
acactctttccctacacgacgctcttccgatct

SEQ ID NO: 4 - DNA, 34 bp, synthetic construct
  source 1..34: mol_type = other DNA
gtgactggagttcagacgtgtgctcttccgatct

SEQ ID NO: 5 - DNA, 30 bp, synthetic construct
  source 1..30: mol_type = other DNA
ccatctcatccctgcgtgtctccgactcag

SEQ ID NO: 6 - DNA, 23 bp, synthetic construct
  source 1..23: mol_type = other DNA
  misc_feature 1..23: note = domains employed on the Ion Torrent-based sequencing platforms
cctctctatgggcagtcggtgat

SEQ ID NO: 7 - DNA, 30 bp, synthetic construct; identical to SEQ ID NO: 5
  source 1..30: mol_type = other DNA
  misc_feature 1..30: note = An exemplary Y-adapter compatible with the Ion Torrent sequencing platform

SEQ ID NO: 8 - DNA, 26 bp, synthetic construct
  source 1..26: mol_type = other DNA
  misc_feature 1..26: note = An exemplary Y-adapter compatible with the Ion Torrent sequencing platform
ccatctcatccctgcgtgtctccgac

SEQ ID NO: 9 - DNA, 28 bp, synthetic construct
  source 1..28: mol_type = other DNA
  misc_feature 1..28: note = An exemplary Y-adapter compatible with the Ion Torrent sequencing platform
ggagagatacccgtcagccactatctga

SEQ ID NO: 10 - DNA, 23 bp, synthetic construct
  source 1..23: mol_type = other DNA
  misc_feature 1..23: note = An exemplary Y-adapter compatible with the Ion Torrent sequencing platform
ggagagatacccgtcagccacta

SEQ ID NO: 11 - DNA, 13 bp, synthetic construct
  source 1..13: mol_type = other DNA
  misc_feature 1..13: note = An exemplary Y-adapter compatible with the Ion Torrent sequencing platform
agcacgaatcgat

SEQ ID NO: 12 - DNA, 12 bp, synthetic construct
  source 1..12: mol_type = other DNA
  misc_feature 1..12: note = An exemplary Y-adapter compatible with the Ion Torrent sequencing platform
tcgtgcttagct

SEQ ID NO: 13 - DNA, 58 bp, synthetic construct
  source 1..58: mol_type = other DNA
aatgatacggcgaccaccgagatctacactctttccctacacgacgctcttccgatct

SEQ ID NO: 14 - DNA, 63 bp, synthetic construct
  source 1..63: mol_type = other DNA
  misc_feature 34..39: note = Each N represents A, C, T or G
gatcggaagagcacacgtctgaactccagtcacnnnnnnatctcgtatgccgtcttctgcttg

SEQ ID NO: 15 - DNA, 51 bp, synthetic construct
  source 1..51: mol_type = other DNA
ggttgtttctgttggtgctgatattgcggcgtctgcttgggtgtttaacct

SEQ ID NO: 16 - DNA, 68 bp, synthetic construct
  source 1..68: mol_type = other DNA
ggttaaacacccaagcagacgccgcaatatcagcaccaacagaaacaacctttgaggcgagcggtcaa

SEQ ID NO: 17 - DNA, 48 bp, synthetic construct
  source 1..48: mol_type = other DNA
  misc_feature 48: note = C bears a C3 spacer which links this C nucleotide to T nucleotide in position 1 in Seq No: 18
cgttctgtttatgtttcttggacactgattgacacggtttagtagaac

SEQ ID NO: 18 - DNA, 49 bp, synthetic construct
  source 1..49: mol_type = other DNA
  misc_feature 1: note = T bears a C3 spacer which links this T nucleotide to C nucleotide in position 48 in Seq No: 17
ttttttttttttttttttttttttttttcaagaaacataaacagaacgt